European Patent Specification EP 4 013 512 B1, published February 14, 2024. Title: BISPECIFIC ANTIBODIES AGAINST CEACAM5 AND CD3. Applicant: LAMKAP BIO ALPHA AG. The sequence listing filed with the application follows.

SEQUENCE LISTING (138 sequences)

SEQ ID NO: 1 - protein, 125 aa, Artificial Sequence
  huCD3 VH
EVQLVESGGGLVQPGGSLKLSCAASGFTFNTYAMNWVRQAPGKGLEWVGRIRSKYNNYATYYADSVKDRFTISRDDSKNTAYLQMNSLKTEDTAVYYCVRHGNFGNSYVSWFAYWGQGTLVTVSS

SEQ ID NO: 2 - protein, 5 aa, Artificial Sequence
  huCD3 CDRH1
TYAMN

SEQ ID NO: 3 - protein, 19 aa, Artificial Sequence
  huCD3 CDRH2
RIRSKYNNYATYYADSVKD

SEQ ID NO: 4 - protein, 14 aa, Artificial Sequence
  huCD3 CDRH3
HGNFGNSYVSWFAY

SEQ ID NO: 5 - protein, 109 aa, Artificial Sequence
  huCD3 VL 1B6
QTVVTQEPSLTVSPGGTVTLTCRSSTGAVTTSNYANWFQQKPGQAPRGLIGGTNKRAPGTPARFSGSLLGGKAALTLSGAQPEDEAEYYCALWYANRWVFGGGTKLTVL

SEQ ID NO: 6 - protein, 14 aa, Artificial Sequence
  huCD3 1B6 CDRL1
RSSTGAVTTSNYAN

SEQ ID NO: 7 - protein, 7 aa, Artificial Sequence
  huCD3 1B6 CDRL2
GTNKRAP

SEQ ID NO: 8 - protein, 9 aa, Artificial Sequence
  huCD3 1B6 CDRL3
ALWYANRWV

SEQ ID NO: 9 - protein, 109 aa, Artificial Sequence
  huCD3 VL 1A10
QTVVTQEPSLTVSPGGTVTLTCRSSTGAVTTSNYANWFQQKPGQAPRGLIGGTNKRAPGTPARFSGSLLGGKAALTLSGAQPEDEAEYYCALWYKGYWVFGGGTKLTVL

SEQ ID NO: 10 - protein, 14 aa, Artificial Sequence
  huCD3 1A10 CDRL1
RSSTGAVTTSNYAN

SEQ ID NO: 11 - protein, 7 aa, Artificial Sequence
  huCD3 1A10 CDRL2
GTNKRAP

SEQ ID NO: 12 - protein, 9 aa, Artificial Sequence
  huCD3 1A10 CDRL3
ALWYKGYWV

SEQ ID NO: 13 - protein, 109 aa, Artificial Sequence
  huCD3 VL 1F8
QTVVTQEPSLTVSPGGTVTLTCRSSTGAVTTSNYANWFQQKPGQAPRGLIGGTNKRAPGTPARFSGSLLGGKAALTLSGAQPEDEAEYYCALWYDGKWVFGGGTKLTVL

SEQ ID NO: 14 - protein, 14 aa, Artificial Sequence
  huCD3 1F8 CDRL1
RSSTGAVTTSNYAN

SEQ ID NO: 15 - protein, 7 aa, Artificial Sequence
  huCD3 1F8 CDRL2
GTNKRAP

SEQ ID NO: 16 - protein, 9 aa, Artificial Sequence
  huCD3 1F8 CDRL3
ALWYDGKWV

SEQ ID NO: 17 - protein, 109 aa, Artificial Sequence
  huCD3 VL 1A4
QTVVTQEPSLTVSPGGTVTLTCRSSTGAVTTSNYANWFQQKPGQAPRGLIGGTNKRAPGTPARFSGSLLGGKAALTLSGAQPEDEAEYYCALWYKQRWVFGGGTKLTVL

SEQ ID NO: 18 - protein, 14 aa, Artificial Sequence
  huCD3 1A4 CDRL1
RSSTGAVTTSNYAN

SEQ ID NO: 19 - protein, 7 aa, Artificial Sequence
  huCD3 1A4 CDRL2
GTNKRAP

SEQ ID NO: 20 - protein, 9 aa, Artificial Sequence
  huCD3 1A4 CDRL3
ALWYKQRWV

SEQ ID NO: 21 - protein, 109 aa, Artificial Sequence
  huCD3 VL 1H4
QTVVTQEPSLTVSPGGTVTLTCRSSTGAVTTSNYANWFQQKPGQAPRGLIGGTNKRAPGTPARFSGSLLGGKAALTLSGAQPEDEAEYYCALWYNQHWVFGGGTKLTVL

SEQ ID NO: 22 - protein, 14 aa, Artificial Sequence
  huCD3 1H4 CDRL1
RSSTGAVTTSNYAN

SEQ ID NO: 23 - protein, 7 aa, Artificial Sequence
  huCD3 1H4 CDRL2
GTNKRAP

SEQ ID NO: 24 - protein, 9 aa, Artificial Sequence
  huCD3 1H4 CDRL3
ALWYNQHWV

SEQ ID NO: 25 - protein, 215 aa, Artificial Sequence
  huCD3 1B6 LC
QTVVTQEPSLTVSPGGTVTLTCRSSTGAVTTSNYANWFQQKPGQAPRGLIGGTNKRAPGTPARFSGSLLGGKAALTLSGAQPEDEAEYYCALWYANRWVFGGGTKLTVLGQPKAAPSVTLFPPSSEELQANKATLVCLISDFYPGAVTVAWKADSSPVKAGVETTTPSKQSNNKYAASSYLSLTPEQWKSHRSYSCQVTHEGSTVEKTVAPTECS

SEQ ID NO: 26 - protein, 215 aa, Artificial Sequence
  huCD3 1A10 LC
QTVVTQEPSLTVSPGGTVTLTCRSSTGAVTTSNYANWFQQKPGQAPRGLIGGTNKRAPGTPARFSGSLLGGKAALTLSGAQPEDEAEYYCALWYKGYWVFGGGTKLTVLGQPKAAPSVTLFPPSSEELQANKATLVCLISDFYPGAVTVAWKADSSPVKAGVETTTPSKQSNNKYAASSYLSLTPEQWKSHRSYSCQVTHEGSTVEKTVAPTECS

SEQ ID NO: 27 - protein, 215 aa, Artificial Sequence
  huCD3 1F8 LC
QTVVTQEPSLTVSPGGTVTLTCRSSTGAVTTSNYANWFQQKPGQAPRGLIGGTNKRAPGTPARFSGSLLGGKAALTLSGAQPEDEAEYYCALWYDGKWVFGGGTKLTVLGQPKAAPSVTLFPPSSEELQANKATLVCLISDFYPGAVTVAWKADSSPVKAGVETTTPSKQSNNKYAASSYLSLTPEQWKSHRSYSCQVTHEGSTVEKTVAPTECS

SEQ ID NO: 28 - protein, 215 aa, Artificial Sequence
  huCD3 1A4 LC
QTVVTQEPSLTVSPGGTVTLTCRSSTGAVTTSNYANWFQQKPGQAPRGLIGGTNKRAPGTPARFSGSLLGGKAALTLSGAQPEDEAEYYCALWYKQRWVFGGGTKLTVLGQPKAAPSVTLFPPSSEELQANKATLVCLISDFYPGAVTVAWKADSSPVKAGVETTTPSKQSNNKYAASSYLSLTPEQWKSHRSYSCQVTHEGSTVEKTVAPTECS

SEQ ID NO: 29 - protein, 215 aa, Artificial Sequence
  huCD3 1H4 LC
QTVVTQEPSLTVSPGGTVTLTCRSSTGAVTTSNYANWFQQKPGQAPRGLIGGTNKRAPGTPARFSGSLLGGKAALTLSGAQPEDEAEYYCALWYNQHWVFGGGTKLTVLGQPKAAPSVTLFPPSSEELQANKATLVCLISDFYPGAVTVAWKADSSPVKAGVETTTPSKQSNNKYAASSYLSLTPEQWKSHRSYSCQVTHEGSTVEKTVAPTECS

SEQ ID NO: 30 - protein, 329 aa, Artificial Sequence
  Common constant heavy chain (WT IgG1)
ASTKGPSVFPLAPSSKSTSGGTAALGCLVKDYFPEPVTVSWNSGALTSGVHTFPAVLQSSGLYSLSSVVTVPSSSLGTQTYICNVNHKPSNTKVDKRVEPKSCDKTHTCPPCPAPELLGGPSVFLFPPKPKDTLMISRTPEVTCVVVDVSHEDPEVKFNWYVDGVEVHNAKTKPREEQYNSTYRVVSVLTVLHQDWLNGKEYKCKVSNKALPAPIEKTISKAKGQPREPQVYTLPPSREEMTKNQVSLTCLVKGFYPSDIAVEWESNGQPENNYKTTPPVLDSDGSFFLYSKLTVDKSRWQQGNVFSCSVMHEALHNHYTQKSLSLSPG

SEQ ID NO: 31 - protein, 109 aa, Artificial Sequence
  CEA VL AB1 (2F2)
EIVLTQSPATLSLSPGERATLSCRASQSVNSNLNWYQQKPGQAPRLLIYHGSNRATGIPARFSGSGSGTDFTLTISSLEPEDFAVYYCQQFDLRHEHNTFGQGTKVEIK

SEQ ID NO: 32 - protein, 11 aa, Artificial Sequence
  CEA AB1 CDRL1
RASQSVNSNLN

SEQ ID NO: 33 - protein, 7 aa, Artificial Sequence
  CEA AB1 CDRL2
HGSNRAT

SEQ ID NO: 34 - protein, 11 aa, Artificial Sequence
  CEA AB1 CDRL3
QQFDLRHEHNT

SEQ ID NO: 35 - protein, 112 aa, Artificial Sequence
  CEA VL AB8 (2A3)
QSALTQPASVSGSPGQSITISCTGTSSDVIENAIVSWYQQHPGKAPKPMIYTLSDRPSGVSNRFSGSKSGNTASLTISGLQAEDEADYYCSSWDTFAIGPAVFGGGTKLTVL

SEQ ID NO: 36 - protein, 14 aa, Artificial Sequence
  CEA AB8 CDRL1
TGTSSDVIENAIVS

SEQ ID NO: 37 - protein, 7 aa, Artificial Sequence
  CEA AB8 CDRL2
TLSDRPS

SEQ ID NO: 38 - protein, 12 aa, Artificial Sequence
  CEA AB8 CDRL3
SSWDTFAIGPAV

SEQ ID NO: 39 - protein, 117 aa, Artificial Sequence
  Constant kappa light chain (CK)
FGQGTKVEIKRTVAAPSVFIFPPSDEQLKSGTASVVCLLNNFYPREAKVQWKVDNALQSGNSQESVTEQDSKDSTYSLSSTLTLSKADYEKHKVYACEVTHQGLSSPVTKSFNRGEC

SEQ ID NO: 40 - protein, 216 aa, Artificial Sequence
  CEA AB1 light chain (VKCK_2F2)
EIVLTQSPATLSLSPGERATLSCRASQSVNSNLNWYQQKPGQAPRLLIYHGSNRATGIPARFSGSGSGTDFTLTISSLEPEDFAVYYCQQFDLRHEHNTFGQGTKVEIKRTVAAPSVFIFPPSDEQLKSGTASVVCLLNNFYPREAKVQWKVDNALQSGNSQESVTEQDSKDSTYSLSSTLTLSKADYEKHKVYACEVTHQGLSSPVTKSFNRGEC

SEQ ID NO: 41 - protein, 116 aa, Artificial Sequence
  Constant lambda light chain (CL)
FGGGTKLTVLGQPKAAPSVTLFPPSSEELQANKATLVCLISDFYPGAVTVAWKADSSPVKAGVETTTPSKQSNNKYAASSYLSLTPEQWKSHRSYSCQVTHEGSTVEKTVAPTECS

SEQ ID NO: 42 - protein, 218 aa, Artificial Sequence
  CEA AB8 light chain (VLCL_2A3)
QSALTQPASVSGSPGQSITISCTGTSSDVIENAIVSWYQQHPGKAPKPMIYTLSDRPSGVSNRFSGSKSGNTASLTISGLQAEDEADYYCSSWDTFAIGPAVFGGGTKLTVLGQPKAAPSVTLFPPSSEELQANKATLVCLISDFYPGAVTVAWKADSSPVKAGVETTTPSKQSNNKYAASSYLSLTPEQWKSHRSYSCQVTHEGSTVEKTVAPTECS

SEQ ID NO: 43 - protein, 454 aa, Artificial Sequence
  Common heavy chain (wild-type)
EVQLVESGGGLVQPGGSLKLSCAASGFTFNTYAMNWVRQAPGKGLEWVGRIRSKYNNYATYYADSVKDRFTISRDDSKNTAYLQMNSLKTEDTAVYYCVRHGNFGNSYVSWFAYWGQGTLVTVSSASTKGPSVFPLAPSSKSTSGGTAALGCLVKDYFPEPVTVSWNSGALTSGVHTFPAVLQSSGLYSLSSVVTVPSSSLGTQTYICNVNHKPSNTKVDKRVEPKSCDKTHTCPPCPAPELLGGPSVFLFPPKPKDTLMISRTPEVTCVVVDVSHEDPEVKFNWYVDGVEVHNAKTKPREEQYNSTYRVVSVLTVLHQDWLNGKEYKCKVSNKALPAPIEKTISKAKGQPREPQVYTLPPSREEMTKNQVSLTCLVKGFYPSDIAVEWESNGQPENNYKTTPPVLDSDGSFFLYSKLTVDKSRWQQGNVFSCSVMHEALHNHYTQKSLSLSPG

SEQ ID NO: 44 - protein, 454 aa, Artificial Sequence
  Common heavy chain (LALA mutation)
EVQLVESGGGLVQPGGSLKLSCAASGFTFNTYAMNWVRQAPGKGLEWVGRIRSKYNNYATYYADSVKDRFTISRDDSKNTAYLQMNSLKTEDTAVYYCVRHGNFGNSYVSWFAYWGQGTLVTVSSASTKGPSVFPLAPSSKSTSGGTAALGCLVKDYFPEPVTVSWNSGALTSGVHTFPAVLQSSGLYSLSSVVTVPSSSLGTQTYICNVNHKPSNTKVDKRVEPKSCDKTHTCPPCPAPEAAGGPSVFLFPPKPKDTLMISRTPEVTCVVVDVSHEDPEVKFNWYVDGVEVHNAKTKPREEQYNSTYRVVSVLTVLHQDWLNGKEYKCKVSNKALPAPIEKTISKAKGQPREPQVYTLPPSREEMTKNQVSLTCLVKGFYPSDIAVEWESNGQPENNYKTTPPVLDSDGSFFLYSKLTVDKSRWQQGNVFSCSVMHEALHNHYTQKSLSLSPG

SEQ ID NO: 45 - protein, 454 aa, Artificial Sequence
  Common heavy chain (LALA+P329A mutation)
EVQLVESGGGLVQPGGSLKLSCAASGFTFNTYAMNWVRQAPGKGLEWVGRIRSKYNNYATYYADSVKDRFTISRDDSKNTAYLQMNSLKTEDTAVYYCVRHGNFGNSYVSWFAYWGQGTLVTVSSASTKGPSVFPLAPSSKSTSGGTAALGCLVKDYFPEPVTVSWNSGALTSGVHTFPAVLQSSGLYSLSSVVTVPSSSLGTQTYICNVNHKPSNTKVDKRVEPKSCDKTHTCPPCPAPEAAGGPSVFLFPPKPKDTLMISRTPEVTCVVVDVSHEDPEVKFNWYVDGVEVHNAKTKPREEQYNSTYRVVSVLTVLHQDWLNGKEYKCKVSNKALAAPIEKTISKAKGQPREPQVYTLPPSREEMTKNQVSLTCLVKGFYPSDIAVEWESNGQPENNYKTTPPVLDSDGSFFLYSKLTVDKSRWQQGNVFSCSVMHEALHNHYTQKSLSLSPG

SEQ ID NO: 46 - protein, 106 aa, Artificial Sequence
  VK_SM3E
ENVLTQSPSSMSVSVGDRVNIACSASSSVPYMHWLQQKPGKSPKLLIYLTSNLASGVPSRFSGSGSGTDYSLTISSVQPEDAATYYCQQRSSYPLTFGGGTKLEIK

SEQ ID NO: 47 - protein, 120 aa, Artificial Sequence
  VH_SM3E
QVKLEQSGAEVVKPGASVKLSCKASGFNIKDSYMHWLRQGPGQRLEWIGWIDPENGDTEYAPKFQGKATFTTDTSANTAYLGLSSLRPEDTAVYYCNEGTPTGPYYFDYWGQGTLVTVSS

SEQ ID NO: 48 - protein, 116 aa, Artificial Sequence
  VL_MEDI
QAVLTQPASLSASPGASASLTCTLRRGINVGAYSIYWYQQKPGSPPQYLLRYKSDSDKQQGSGVSSRFSASKDASANAGILLISGLQSEDEADYYCMIWHSGASAVFGGGTKLTVL

SEQ ID NO: 49 - protein, 121 aa, Artificial Sequence
  VH_MEDI
EVQLVESGGGLVQPGRSLRLSCAASGFTVSSYWMHWVRQAPGKGLEWVGFIRNKANGGTTEYAASVKGRFTISRDDSKNTLYLQMNSLRAEDTAVYYCARDRGLRFYFDYWGQGTTVTVSS

SEQ ID NO: 50 - protein, 107 aa, Artificial Sequence
  VK_SAR
DIQMTQSPSSLSASVGDRVTITCRASENIFSYLAWYQQKPGKAPKLLIYNTRTLQSGVPSRFSGSGSGTDFTLTISSLQPEDFATYYCQHHYGTPFTFGQGTKLEIK

SEQ ID NO: 51 - protein, 120 aa, Artificial Sequence
  VH_SAR
EVQLVESGGGLVQPGGSLRLSCAASGFVFSSYDMSWVRQAPGKGLEWVSYISSGGGITYYADSVKGRFTISRDNSKNTLYLQMNSLRAEDTAVYYCAAHYFGSSGPFAYWGQGTLVTVSS

SEQ ID NO: 52 - protein, 108 aa, Artificial Sequence
  VK_CH1A1A
DIQMTQSPSSLSASVGDRVTITCKASAAVGTYVAWYQQKPGKAPKLLIYSASYRKRGVPSRFSGSGSGTDFTLTISSLQPEDFATYYCHQYYTYPLFTFGQGTKLEIK

SEQ ID NO: 53 - protein, 121 aa, Artificial Sequence
  VH_ CH1A1A
QVQLVQSGAEVKKPGASVKVSCKASGYTFTEFGMNWVRQAPGQGLEWMGWINTKTGEATYVEEFKGRVTFTTDTSTSTAYMELRSLRSDDTAVYYCARWDFAYYVEAMDYWGQGTTVTVSS

SEQ ID NO: 54 - protein, 111 aa, Artificial Sequence
  VK_T84.66
EIVLTQSPATLSLSPGERATLSCRAGESVDIFGVGFLHWYQQKPGQAPRLLIYRASNRATGIPARFSGSGSGTDFTLTISSLEPEDFAVYYCQQTNEDPYTFGQGTKLEIK

SEQ ID NO: 55 - protein, 121 aa, Artificial Sequence
  VH_T84.66
QVQLVQSGAEVKKPGSSVKVSCKASGFNIKDTYMHWVRQAPGQGLEWMGRIDPANGNSKYVPKFQGRVTITADTSTSTAYMELSSLRSEDTAVYYCAPFGYYVSDYAMAYWGQGTLVTVSS

SEQ ID NO: 56 - protein, 106 aa, Artificial Sequence
  VK_LABETUZUMAB
DIQLTQSPSSLSASVGDRVTITCKASQDVGTSVAWYQQKPGKAPKLLIYWTSTRHTGVPSRFSGSGSGTDFTFTISSLQPEDIATYYCQQYSLYRSFGQGTKVEIK

SEQ ID NO: 57 - protein, 119 aa, Artificial Sequence
  VH_LABETUZUMAB
EVQLVESGGGVVQPGRSLRLSCSASGFDFTTYWMSWVRQAPGKGLEWIGEIHPDSSTINYAPSLKDRFTISRDNAKNTLFLQMDSLRPEDTGVYFCASLYFGFPWFAYWGQGTPVTVSS

SEQ ID NO: 58 - protein, 118 aa, Artificial Sequence
  Constant hybrid-kappa light chain (H-CK 5)
FGGGTKLTVLGRTVAAPSVFIFPPSDEQLKSGTASVVCLLNNFYPREAKVQWKVDNALQSGNSQESVTEQDSKDSTYSLSSTLTLSKADYEKHKVYACEVTHQGLSSPVTKSFNRGEC

SEQ ID NO: 59 - protein, 110 aa, Artificial Sequence
  CEA VL 1B4
SYVLTQPPSVSVAPGKTARITCGGNLIGKNAVHWYQQKPGQAPVLVIYNYGIRPSGIPERFSGSNSGNTATLTISRVEAGDEADYYCQVWDTLKLEPDAVFGGGTKLTVL

SEQ ID NO: 60 - protein, 11 aa, Artificial Sequence
  CEA 1B4 CDRL1
GGNLIGKNAVH

SEQ ID NO: 61 - protein, 7 aa, Artificial Sequence
  CEA 1B4 CDRL2
NYGIRPS

SEQ ID NO: 62 - protein, 13 aa, Artificial Sequence
  CEA 1B4 CDRL3
QVWDTLKLEPDAV

SEQ ID NO: 63 - protein, 107 aa, Artificial Sequence
  CEA VL C11
DIQMTQSPSTLSASVGDRVTITCRASQLISNGLYWYQQKPGKAPKLLIYDASILESGVPSRFSGSGSGTEFTLTISSLQPDDFATYYCQQRLSWPLTFGQGTKVEIK

SEQ ID NO: 64 - protein, 11 aa, Artificial Sequence
  CEA C11 CDRL1
RASQLISNGLY

SEQ ID NO: 65 - protein, 7 aa, Artificial Sequence
  CEA C11 CDRL2
DASILES

SEQ ID NO: 66 - protein, 9 aa, Artificial Sequence
  CEA C11 CDRL3
QQRLSWPLT

SEQ ID NO: 67 - protein, 217 aa, Artificial Sequence
  huCD3 1B6 LC-hybrid kappa
QTVVTQEPSLTVSPGGTVTLTCRSSTGAVTTSNYANWFQQKPGQAPRGLIGGTNKRAPGTPARFSGSLLGGKAALTLSGAQPEDEAEYYCALWYANRWVFGGGTKLTVLGRTVAAPSVFIFPPSDEQLKSGTASVVCLLNNFYPREAKVQWKVDNALQSGNSQESVTEQDSKDSTYSLSSTLTLSKADYEKHKVYACEVTHQGLSSPVTKSFNRGEC

SEQ ID NO: 68 - protein, 217 aa, Artificial Sequence
  huCD3 1A10 LC-hybrid kappa
QTVVTQEPSLTVSPGGTVTLTCRSSTGAVTTSNYANWFQQKPGQAPRGLIGGTNKRAPGTPARFSGSLLGGKAALTLSGAQPEDEAEYYCALWYKGYWVFGGGTKLTVLGRTVAAPSVFIFPPSDEQLKSGTASVVCLLNNFYPREAKVQWKVDNALQSGNSQESVTEQDSKDSTYSLSSTLTLSKADYEKHKVYACEVTHQGLSSPVTKSFNRGEC

SEQ ID NO: 69 - protein, 217 aa, Artificial Sequence
  huCD3 1F8 LC-hybrid kappa
QTVVTQEPSLTVSPGGTVTLTCRSSTGAVTTSNYANWFQQKPGQAPRGLIGGTNKRAPGTPARFSGSLLGGKAALTLSGAQPEDEAEYYCALWYDGKWVFGGGTKLTVLGRTVAAPSVFIFPPSDEQLKSGTASVVCLLNNFYPREAKVQWKVDNALQSGNSQESVTEQDSKDSTYSLSSTLTLSKADYEKHKVYACEVTHQGLSSPVTKSFNRGEC

SEQ ID NO: 70 - protein, 217 aa, Artificial Sequence
  huCD3 1A4 LC-hybrid kappa
QTVVTQEPSLTVSPGGTVTLTCRSSTGAVTTSNYANWFQQKPGQAPRGLIGGTNKRAPGTPARFSGSLLGGKAALTLSGAQPEDEAEYYCALWYKQRWVFGGGTKLTVLGRTVAAPSVFIFPPSDEQLKSGTASVVCLLNNFYPREAKVQWKVDNALQSGNSQESVTEQDSKDSTYSLSSTLTLSKADYEKHKVYACEVTHQGLSSPVTKSFNRGEC

SEQ ID NO: 71 - protein, 217 aa, Artificial Sequence
  huCD3 1H4 LC-hybrid kappa
QTVVTQEPSLTVSPGGTVTLTCRSSTGAVTTSNYANWFQQKPGQAPRGLIGGTNKRAPGTPARFSGSLLGGKAALTLSGAQPEDEAEYYCALWYNQHWVFGGGTKLTVLGRTVAAPSVFIFPPSDEQLKSGTASVVCLLNNFYPREAKVQWKVDNALQSGNSQESVTEQDSKDSTYSLSSTLTLSKADYEKHKVYACEVTHQGLSSPVTKSFNRGEC

SEQ ID NO: 72 - protein, 220 aa, Artificial Sequence
  CEA 2A3 LC-hybrid kappa
QSALTQPASVSGSPGQSITISCTGTSSDVIENAIVSWYQQHPGKAPKPMIYTLSDRPSGVSNRFSGSKSGNTASLTISGLQAEDEADYYCSSWDTFAIGPAVFGGGTKLTVLGRTVAAPSVFIFPPSDEQLKSGTASVVCLLNNFYPREAKVQWKVDNALQSGNSQESVTEQDSKDSTYSLSSTLTLSKADYEKHKVYACEVTHQGLSSPVTKSFNRGEC

SEQ ID NO: 73 - protein, 214 aa, Artificial Sequence
  CEA C11 LC (VKCK_C11)
DIQMTQSPSTLSASVGDRVTITCRASQLISNGLYWYQQKPGKAPKLLIYDASILESGVPSRFSGSGSGTEFTLTISSLQPDDFATYYCQQRLSWPLTFGQGTKVEIKRTVAAPSVFIFPPSDEQLKSGTASVVCLLNNFYPREAKVQWKVDNALQSGNSQESVTEQDSKDSTYSLSSTLTLSKADYEKHKVYACEVTHQGLSSPVTKSFNRGEC

SEQ ID NO: 74 - protein, 216 aa, Artificial Sequence
  CEA 1B4 LCEA 1B4 LC (VLCL_1B4)
SYVLTQPPSVSVAPGKTARITCGGNLIGKNAVHWYQQKPGQAPVLVIYNYGIRPSGIPERFSGSNSGNTATLTISRVEAGDEADYYCQVWDTLKLEPDAVFGGGTKLTVLGQPKAAPSVTLFPPSSEELQANKATLVCLISDFYPGAVTVAWKADSSPVKAGVETTTPSKQSNNKYAASSYLSLTPEQWKSHRSYSCQVTHEGSTVEKTVAPTECS

SEQ ID NO: 75 - protein, 218 aa, Artificial Sequence
  CEA 1B4 LC-hybrid kappa (VLCK_1B4)
SYVLTQPPSVSVAPGKTARITCGGNLIGKNAVHWYQQKPGQAPVLVIYNYGIRPSGIPERFSGSNSGNTATLTISRVEAGDEADYYCQVWDTLKLEPDAVFGGGTKLTVLGRTVAAPSVFIFPPSDEQLKSGTASVVCLLNNFYPREAKVQWKVDNALQSGNSQESVTEQDSKDSTYSLSSTLTLSKADYEKHKVYACEVTHQGLSSPVTKSFNRGEC

SEQ ID NO: 76 - DNA, 645 bp, Artificial Sequence
  VKCK_C11 (DNA)
gacatccagatgacccagtctccttccaccctgtctgcatctgtaggagacagagtcaccatcacttgccgggccagtcagcttattagtaatggtttgtattggtatcagcagaaaccagggaaagcccctaagctcctgatctatgatgcttccattttggaaagtggggtcccatcaaggttcagcggcagtggatctgggacagagttcactctcaccatcagcagcctgcagcctgatgattttgcaacttattactgtcagcagcgtctcagctggcctctcactttcggccaagggaccaaggtggaaatcaaacgtacggtggctgcaccatctgtcttcatcttcccgccatctgatgagcagttgaaatctggaactgcctctgttgtgtgcctgctgaataacttctatcccagagaggccaaagtacagtggaaggtggataacgccctccaatcgggtaactcccaggagagtgtcacagagcaggacagcaaggacagcacctacagcctcagcagcaccctgacgctgagcaaagcagactacgagaaacacaaagtctacgcctgcgaagtcacccatcagggcctgagctcgcccgtcacaaagagcttcaacaggggagagtgttaa

SEQ ID NO: 77 - DNA, 651 bp, Artificial Sequence
  VLCL_1B4 (DNA)
tcctatgtgctgactcagccaccctcagtgtcagtggccccaggaaagacggccaggattacctgtgggggaaaccttattggaaagaatgctgtgcactggtaccagcagaagccaggccaggcccctgtgctggtcatctataattatggtattcggccctcagggattcctgagcgattctctggctccaactctgggaacacggccaccctgaccatcagcagggtcgaagccggggatgaggccgactattactgtcaggtgtgggatactcttaagcttgagcctgatgctgtgttcggcggagggaccaagctgaccgtcctaggtcagcccaaggctgccccctcggtcactctgttcccgccctcctctgaggagcttcaagccaacaaggccacactggtgtgtctcataagtgacttctacccgggagccgtgacagtggcttggaaagcagatagcagccccgtcaaggcgggagtggagaccaccacaccctccaaacaaagcaacaacaagtacgcggccagcagctatctgagcctgacgcctgagcagtggaagtcccacagaagctacagctgccaggtcacgcatgaagggagcaccgtggagaagacagtggcccctacagaatgttcataa

SEQ ID NO: 78 - DNA, 651 bp, Artificial Sequence
  VKCK_2F2 (AB1) (DNA)
gaaattgtgttgacacagtctccagccaccctgtctttgtctccaggggaaagagccaccctctcctgcagggccagtcagtctgttaattctaatttaaattggtaccaacagaaacctggccaggctcccaggctcctcatctatcatgggtccaatagggccactggcatcccagccaggttcagtggcagtgggtctgggacagacttcactctcaccatcagcagcctagagcctgaagattttgcagtttattactgtcagcagtttgatcttaggcatgagcataataccttcggccaagggaccaaggtggaaatcaaacgtacggtggctgcaccatctgtcttcatcttcccgccatctgatgagcagttgaaatctggaactgcctctgttgtgtgcctgctgaataacttctatcccagagaggccaaagtacagtggaaggtggataacgccctccaatcgggtaactcccaggagagtgtcacagagcaggacagcaaggacagcacctacagcctcagcagcaccctgacgctgagcaaagcagactacgagaaacacaaagtctacgcctgcgaagtcacccatcagggcctgagctcgcccgtcacaaagagcttcaacaggggagagtgttaa

SEQ ID NO: 79 - DNA, 657 bp, Artificial Sequence
  VLCL_2A3 (AB8) (DNA)
cagtctgccctgactcagcctgcctccgtgtctgggtctcctggacagtcgatcaccatctcctgcactggaaccagcagtgacgttattgagaatgctattgtctcctggtaccaacagcacccaggcaaagcccccaaacccatgatttatactcttagtgatcggccctcaggggtttctaatcgcttctctggctccaagtctggcaacacggcctccctgaccatctctgggctccaggctgaggacgaggctgattattactgcagctcatgggatacttttgcgattggtcctgctgtgttcggcggagggaccaagctgaccgtcctaggtcagcccaaggctgccccctcggtcactctgttcccgccctcctctgaggagcttcaagccaacaaggccacactggtgtgtctcataagtgacttctacccgggagccgtgacagtggcttggaaagcagatagcagccccgtcaaggcgggagtggagaccaccacaccctccaaacaaagcaacaacaagtacgcggccagcagctatctgagcctgacgcctgagcagtggaagtcccacagaagctacagctgccaggtcacgcatgaagggagcaccgtggagaagacagtggcccctacagaatgttcataa

SEQ ID NO: 80 - DNA, 1365 bp, Artificial Sequence
  Common heavy chain VHCH (wild-type; DNA)
gaggtgcagctggtggagtctgggggaggcttggtccagcctggggggtccctgaaactctcctgtgcagcctctgggttcaccttcaacacctatgctatgaactgggtccgccaggctcccgggaaagggctggagtgggttggccgtattagaagcaaatataacaattacgcgacatactatgctgactcggtgaaagacaggttcaccatctccagagatgattcaaagaacacggcgtatctgcaaatgaacagcctgaaaaccgaggacacggccgtgtattactgtgtgagacacgggaatttcggcaattcttatgtctcgtggttcgcttactggggccaagggactctggtcacagtctcgagcgcctccaccaagggcccatcggtcttccccctggcaccctcctccaagagcacctctgggggcacagcggccctgggctgcctggtcaaggactacttccccgaaccggtgacagtctcgtggaactcaggagccctgaccagcggcgtgcacaccttcccggctgtcctacagtcctcaggactctactccctcagcagcgtggtgactgtgccctccagcagcttgggcacccagacctacatctgcaacgtgaatcacaagcccagcaacaccaaggtggacaagagagttgagcccaaatcttgtgacaaaactcacacatgcccaccgtgcccagcacctgaactcctggggggaccgtcagtcttcctcttccccccaaaacccaaggacaccctcatgatctcccggacccctgaggtcacatgcgtggtggtggacgtgagccacgaagaccctgaggtcaagttcaactggtacgtggacggcgtggaggtgcataatgccaagacaaagccgcgggaggagcagtacaacagcacgtaccgtgtggtcagcgtcctcaccgtcctgcaccaggactggctgaatggcaaggagtacaagtgcaaggtctccaacaaagccctcccagcccccatcgagaaaaccatctccaaagccaaagggcagccccgagaaccacaggtgtataccctgcccccatctcgggaggagatgaccaagaaccaggtcagcctgacttgcctggtcaaaggcttctatcccagcgacatcgccgtggagtgggagagcaacgggcagccggagaacaactacaagaccacgcctcccgtgctggactccgacggctccttcttcctctatagcaagctcaccgtggacaagtccaggtggcagcaggggaacgtcttctcatgctccgtgatgcatgaggctctgcacaaccactacacgcagaagagcctctccctgtctccgggttaa

SEQ ID NO: 81 - protein, 11 aa, Artificial Sequence
  CEA AB13 CDRL1
RASQSVNSNLN

SEQ ID NO: 82 - protein, 7 aa, Artificial Sequence
  CEA AB13 CDRL2
HGSNRAT

SEQ ID NO: 83 - protein, 11 aa, Artificial Sequence
  CEA AB13 CDRL3
QQFDYFMNKNT

SEQ ID NO: 84 - protein, 11 aa, Artificial Sequence
  CEA AB14 CDRL1
RASQSVNSNLN

SEQ ID NO: 85 - protein, 7 aa, Artificial Sequence
  CEA AB14 CDRL2
HGSNRAT

SEQ ID NO: 86 - protein, 11 aa, Artificial Sequence
  CEA AB14 CDRL3
QQFDYFRESNT

SEQ ID NO: 87 - protein, 11 aa, Artificial Sequence
  CEA AB15 CDRL1
RASQTVNNNLN

SEQ ID NO: 88 - protein, 7 aa, Artificial Sequence
  CEA AB15 CDRL2
YASNRAT

SEQ ID NO: 89 - protein, 11 aa, Artificial Sequence
  CEA AB15 CDRL3
QQFNYHHEHNT

SEQ ID NO: 90 - protein, 11 aa, Artificial Sequence
  CEA AB17 CDRL1
RASQSVNSNLN

SEQ ID NO: 91 - protein, 7 aa, Artificial Sequence
  CEA AB17 CDRL2
HGSNRAT

SEQ ID NO: 92 - protein, 11 aa, Artificial Sequence
  CEA AB17 CDRL3
QQFDYFKEHNT

SEQ ID NO: 93 - protein, 11 aa, Artificial Sequence
  CEA AB20 CDRL1
RASQSVNSNLN

SEQ ID NO: 94 - protein, 7 aa, Artificial Sequence
  CEA AB20 CDRL2
HGSNRAT

SEQ ID NO: 95 - protein, 11 aa, Artificial Sequence
  CEA AB20 CDRL3
QQFDYFRELNT

SEQ ID NO: 96 - protein, 11 aa, Artificial Sequence
  CEA AB54 CDRL1
RASQEVHKNLN

SEQ ID NO: 97 - protein, 7 aa, Artificial Sequence
  CEA AB54 CDRL2
HSSNRAT

SEQ ID NO: 98 - protein, 11 aa, Artificial Sequence
  CEA AB54 CDRL3
QQFNYHHEHNT

SEQ ID NO: 99 - protein, 11 aa, Artificial Sequence
  CEA AB60 CDRL1
RASQTVNANLN

SEQ ID NO: 100 - protein, 7 aa, Artificial Sequence
  CEA AB60 CDRL2
YASNRAT

SEQ ID NO: 101 - protein, 11 aa, Artificial Sequence
  CEA AB60 CDRL3
QQFDYHNEHNT

SEQ ID NO: 102 - protein, 11 aa, Artificial Sequence
  CEA AB66 CDRL1
HSSQVVNKNLN

SEQ ID NO: 103 - protein, 7 aa, Artificial Sequence
  CEA AB66 CDRL2
HGSNRAT

SEQ ID NO: 104 - protein, 11 aa, Artificial Sequence
  CEA AB66 CDRL3
QQFDYFREHNT

SEQ ID NO: 105 - protein, 11 aa, Artificial Sequence
  CEA AB71 CDRL1
RASQSVNSNLN

SEQ ID NO: 106 - protein, 7 aa, Artificial Sequence
  CEA AB71 CDRL2
HSSNRPH

SEQ ID NO: 107 - protein, 11 aa, Artificial Sequence
  CEA AB71 CDRL3
QQFDYFKEHNT

SEQ ID NO: 108 - protein, 11 aa, Artificial Sequence
  CEA AB72 CDRL1
RASQSVNSNLN

SEQ ID NO: 109 - protein, 7 aa, Artificial Sequence
  CEA AB72 CDRL2
HSTNRPR

SEQ ID NO: 110 - protein, 11 aa, Artificial Sequence
  CEA AB72 CDRL3
QQFDYFKEYNT

SEQ ID NO: 111 - protein, 11 aa, Artificial Sequence
  CEA AB73 CDRL1
RASQSVNSNLN

SEQ ID NO: 112 - protein, 7 aa, Artificial Sequence
  CEA AB73 CDRL2
HSNNRPH

SEQ ID NO: 113 - protein, 11 aa, Artificial Sequence
  CEA AB73 CDRL3
QQFDYFREYNT

SEQ ID NO: 114 - protein, 109 aa, Artificial Sequence
  CEA AB13 VL variable light chain region
EIVLTQSPATLSLSPGERATLSCRASQSVNSNLNWYQQKPGQAPRLLIYHGSNRATGIPARFSGSGSGTDFTLTISSLEPEDFAVYYCQQFDYFMNKNTFGQGTKVEIK

SEQ ID NO: 115 - protein, 109 aa, Artificial Sequence
  CEA AB14 VL variable light chain region
EIVLTQSPATLSLSPGERATLSCRASQTVNNNLNWYQQKPGQSPRLLIYYASNRATGIPARFSGSGSGTDFTLTISSLEPEDFAVYYCQQFNYHHEHNTFGQGTKVEIK

SEQ ID NO: 116 - protein, 109 aa, Artificial Sequence; identical to SEQ ID NO: 115
  CEA AB15 VL variable light chain region

SEQ ID NO: 117 - protein, 109 aa, Artificial Sequence
  CEA AB17 VL variable light chain region
EIVLTQSPATLSLSPGERATLSCRASQSVNSNLNWYQQKPGQAPRLLIYHGSNRATGIPARFSGSGSGTDFTLTISSLEPEDFAVYYCQQFDYFKEHNTFGQGTKVEIK

SEQ ID NO: 118 - protein, 109 aa, Artificial Sequence
  CEA AB20 VL variable light chain region
EIVLTQSPATLSLSPGERATLSCRASQSVNSNLNWYQQKPGQAPRLLIYHGSNRATGIPARFSGSGSGTDFTLTISSLEPEDFAVYYCQQFDYFRELNTFGQGTKVEIK

SEQ ID NO: 119 - protein, 109 aa, Artificial Sequence
  CEA AB54 VL variable light chain region
EIVLTQSPATLSLSPGERATLSCRASQEVHKNLNWYQQKPGQAPRLLIYHSSNRATGIPARFSGSGSGTDFTLTISSLEPEDFAVYYCQQFNYHHEHNTFGQGTKVEIK

SEQ ID NO: 120 - protein, 109 aa, Artificial Sequence
  CEA AB60 VL variable light chain region
EIVLTQSPATLSLSPGERATLSCRASQTVNANLNWYQQKPGQAPRLLIYYASNRATGIPARFSGSGSGTDFTLTISSLEPEDFAVYYCQQFDYHNEHNTFGQGTKVEIK

SEQ ID NO: 121 - protein, 109 aa, Artificial Sequence
  CEA AB66 VL variable light chain region
EIVLTQSPATLSLSPGERATLSCHSSQVVNKNLNWYQQKPGQAPRLLIYHGSNRATGIPARFSGSGSGTDFTLTISSLEPEDFAVYYCQQFDYFREHNTFGQGTKVEIK

SEQ ID NO: 122 - protein, 109 aa, Artificial Sequence
  CEA AB71 VL variable light chain region
EIVLTQSPATLSLSPGERATLSCRASQSVNSNLNWYQQKPGQAPRLLIYHSSNRPHGIPARFSGSGSGTDFTLTISSLEPEDFAVYYCQQFDYFKEHNTFGQGTKVEIK

SEQ ID NO: 123 - protein, 109 aa, Artificial Sequence
  CEA AB72 VL variable light chain region
EIVLTQSPATLSLSPGERATLSCRASQSVNSNLNWYQQKPGQAPRLLIYHSTNRPRGIPARFSGSGSGTDFTLTISSLEPEDFAVYYCQQFDYFKEYNTFGQGTKVEIK

SEQ ID NO: 124 - protein, 109 aa, Artificial Sequence
  CEA AB73 VL variable light chain region
EIVLTQSPATLSLSPGERATLSCRASQSVNSNLNWYQQKPGQAPRLLIYHSNNRPHGIPARFSGSGSGTDFTLTISSLEPEDFAVYYCQQFDYFREYNTFGQGTKVEIK

SEQ ID NO: 125 - protein, 216 aa, Artificial Sequence
  CEA AB13 LC light chain
EIVLTQSPATLSLSPGERATLSCRASQSVNSNLNWYQQKPGQAPRLLIYHGSNRATGIPARFSGSGSGTDFTLTISSLEPEDFAVYYCQQFDYFMNKNTFGQGTKVEIKRTVAAPSVFIFPPSDEQLKSGTASVVCLLNNFYPREAKVQWKVDNALQSGNSQESVTEQDSKDSTYSLSSTLTLSKADYEKHKVYACEVTHQGLSSPVTKSFNRGEC

SEQ ID NO: 126 - protein, 216 aa, Artificial Sequence
  CEA AB14 LC light chain
EIVLTQSPATLSLSPGERATLSCRASQSVNSNLNWYQQKPGQAPRLLIYHGSNRATGIPARFSGSGSGTDFTLTISSLEPEDFAVYYCQQFDYFRESNTFGQGTKVEIKRTVAAPSVFIFPPSDEQLKSGTASVVCLLNNFYPREAKVQWKVDNALQSGNSQESVTEQDSKDSTYSLSSTLTLSKADYEKHKVYACEVTHQGLSSPVTKSFNRGEC

SEQ ID NO: 127 - protein, 216 aa, Artificial Sequence
  CEA AB15 LC light chain
EIVLTQSPATLSLSPGERATLSCRASQTVNNNLNWYQQKPGQSPRLLIYYASNRATGIPARFSGSGSGTDFTLTISSLEPEDFAVYYCQQFNYHHEHNTFGQGTKVEIKRTVAAPSVFIFPPSDEQLKSGTASVVCLLNNFYPREAKVQWKVDNALQSGNSQESVTEQDSKDSTYSLSSTLTLSKADYEKHKVYACEVTHQGLSSPVTKSFNRGEC

SEQ ID NO: 128 - protein, 216 aa, Artificial Sequence
  CEA AB17 LC light chain
EIVLTQSPATLSLSPGERATLSCRASQSVNSNLNWYQQKPGQAPRLLIYHGSNRATGIPARFSGSGSGTDFTLTISSLEPEDFAVYYCQQFDYFKEHNTFGQGTKVEIKRTVAAPSVFIFPPSDEQLKSGTASVVCLLNNFYPREAKVQWKVDNALQSGNSQESVTEQDSKDSTYSLSSTLTLSKADYEKHKVYACEVTHQGLSSPVTKSFNRGEC

SEQ ID NO: 129 - protein, 216 aa, Artificial Sequence
  CEA AB20 LC light chain
EIVLTQSPATLSLSPGERATLSCRASQSVNSNLNWYQQKPGQAPRLLIYHGSNRATGIPARFSGSGSGTDFTLTISSLEPEDFAVYYCQQFDYFRELNTFGQGTKVEIKRTVAAPSVFIFPPSDEQLKSGTASVVCLLNNFYPREAKVQWKVDNALQSGNSQESVTEQDSKDSTYSLSSTLTLSKADYEKHKVYACEVTHQGLSSPVTKSFNRGEC

SEQ ID NO: 130 - protein, 216 aa, Artificial Sequence
  CEA AB54 LC light chain
EIVLTQSPATLSLSPGERATLSCRASQEVHKNLNWYQQKPGQAPRLLIYHSSNRATGIPARFSGSGSGTDFTLTISSLEPEDFAVYYCQQFNYHHEHNTFGQGTKVEIKRTVAAPSVFIFPPSDEQLKSGTASVVCLLNNFYPREAKVQWKVDNALQSGNSQESVTEQDSKDSTYSLSSTLTLSKADYEKHKVYACEVTHQGLSSPVTKSFNRGEC

SEQ ID NO: 131 - protein, 216 aa, Artificial Sequence
  CEA AB60 LC light chain
EIVLTQSPATLSLSPGERATLSCRASQTVNANLNWYQQKPGQAPRLLIYYASNRATGIPARFSGSGSGTDFTLTISSLEPEDFAVYYCQQFDYHNEHNTFGQGTKVEIKRTVAAPSVFIFPPSDEQLKSGTASVVCLLNNFYPREAKVQWKVDNALQSGNSQESVTEQDSKDSTYSLSSTLTLSKADYEKHKVYACEVTHQGLSSPVTKSFNRGEC

SEQ ID NO: 132 - protein, 216 aa, Artificial Sequence
  CEA AB66 LC light chain
EIVLTQSPATLSLSPGERATLSCHSSQVVNKNLNWYQQKPGQAPRLLIYHGSNRATGIPARFSGSGSGTDFTLTISSLEPEDFAVYYCQQFDYFREHNTFGQGTKVEIKRTVAAPSVFIFPPSDEQLKSGTASVVCLLNNFYPREAKVQWKVDNALQSGNSQESVTEQDSKDSTYSLSSTLTLSKADYEKHKVYACEVTHQGLSSPVTKSFNRGEC

SEQ ID NO: 133 - protein, 216 aa, Artificial Sequence
  CEA AB71 LC light chain
EIVLTQSPATLSLSPGERATLSCRASQSVNSNLNWYQQKPGQAPRLLIYHSSNRPHGIPARFSGSGSGTDFTLTISSLEPEDFAVYYCQQFDYFKEHNTFGQGTKVEIKRTVAAPSVFIFPPSDEQLKSGTASVVCLLNNFYPREAKVQWKVDNALQSGNSQESVTEQDSKDSTYSLSSTLTLSKADYEKHKVYACEVTHQGLSSPVTKSFNRGEC

SEQ ID NO: 134 - protein, 216 aa, Artificial Sequence
  CEA AB72 LC light chain
EIVLTQSPATLSLSPGERATLSCRASQSVNSNLNWYQQKPGQAPRLLIYHSTNRPRGIPARFSGSGSGTDFTLTISSLEPEDFAVYYCQQFDYFKEYNTFGQGTKVEIKRTVAAPSVFIFPPSDEQLKSGTASVVCLLNNFYPREAKVQWKVDNALQSGNSQESVTEQDSKDSTYSLSSTLTLSKADYEKHKVYACEVTHQGLSSPVTKSFNRGEC

SEQ ID NO: 135 - protein, 216 aa, Artificial Sequence
  CEA AB73 LC light chain
EIVLTQSPATLSLSPGERATLSCRASQSVNSNLNWYQQKPGQAPRLLIYHSNNRPHGIPARFSGSGSGTDFTLTISSLEPEDFAVYYCQQFDYFREYNTFGQGTKVEIKRTVAAPSVFIFPPSDEQLKSGTASVVCLLNNFYPREAKVQWKVDNALQSGNSQESVTEQDSKDSTYSLSSTLTLSKADYEKHKVYACEVTHQGLSSPVTKSFNRGEC

SEQ ID NO: 136 - protein, 11 aa, Artificial Sequence
  CEA AB1 CDRL1 mutation
  misc_feature (1)..(2): Xaa can be any naturally occurring amino acid
  misc_feature (5)..(5): Xaa can be any naturally occurring amino acid
  misc_feature (7)..(8): Xaa can be any naturally occurring amino acid
XXSQXVXXNLN

SEQ ID NO: 137 - protein, 7 aa, Artificial Sequence
  CEA AB1 CDRL2 mutation
  misc_feature (1)..(3): Xaa can be any naturally occurring amino acid
  misc_feature (6)..(7): Xaa can be any naturally occurring amino acid
XXXNRXX

SEQ ID NO: 138 - protein, 11 aa, Artificial Sequence
  CEA AB1 CDRL3 mutation
  misc_feature (2)..(2): Xaa can be any naturally occurring amino acid
  misc_feature (4)..(7): Xaa can be any naturally occurring amino acid
  misc_feature (9)..(9): Xaa can be any naturally occurring amino acid
QXFXXXXEXNT